European Patent Application EP 4 692 112 A2, published February 11, 2026. Title: RECOMBINANT ENGINEERING BACTERIUM FOR PREPARING RECOMBINANT ALBUMIN AND USE THEREOF. Applicant: Tonghua Anrate Biopharmaceutical Co., Ltd. The sequence listing filed with the application follows.

SEQUENCE LISTING (34 sequences)

SEQ ID NO: 1 - DNA, 1047 bp, artificial
  source 1..1047: mol_type = genomic DNA
atgcaagttaaatctatcgttaacctactgttggcatgttcgttggccgtggccagacctttggagcacgcccaccatcaacatgacaagagaggtgttgtcgtcgtgaccaagaccatcgttgtcgatggttccaccgttgaggctaccgcagcagcccaggtccaagagcacgctgaaactttcgcagagtcgactccttcagctgttgtttccagttcatcagctccttcctctgcttcttctgcttccgctcctgcctcttccggtagcttctccgctggaaccaaaggtgtcacctactctccttaccaagccggtggtggctgtaagactgcagaggaggtcgcttccgatctttcccagttgaccggctacgagatcatcagattgtacggtgttgactgtaaccaagtcgagaacgtcttcaaggccaaggccccaggtcaaaagttgtttttgggaatcttctttgttgatgctatcgagagcggtgtcagtgctattgcctccgctgtcaagtcatacggttcttgggacgatgtccacactgtctctgttggtaacgagttggtcaacaacggtgaggccactgtttcccaaatcggtcaatacgtttctaccgctaaatctgccttgagatctgctggtttcaccggtccagttctttctgtcgacactttcattgctgtcatcaacaacccagggttgtgtgactttgctgacgagtacgttgccgttaacgctcacgctttctttgacggtggcattgctgcctctggagctggtgattgggctgctgagcagatccaaagagtttcttccgcttgtggtggcaaggatgtcctcattgtcgagtccggatggccttcaaagggagacaccaacggtgctgccgttccttccaagtcaaaccaacaggctgctgtccaatctctaggtcagaagatcggttcttcttgtattgctttcaacgctttcaacgattactggaaggccgatggtcctttcaacgctgagaagtactggggtatcctagactcctaa

SEQ ID NO: 2 - protein, 348 aa, pichia pastoris
MQVKSIVNLLLACSLAVARPLEHAHHQHDKRGVVVVTKTIVVDGSTVEATAAAQVQEHAETFAESTPSAVVSSSSAPSSASSASAPASSGSFSAGTKGVTYSPYQAGGGCKTAEEVASDLSQLTGYEIIRLYGVDCNQVENVFKAKAPGQKLFLGIFFVDAIESGVSAIASAVKSYGSWDDVHTVSVGNELVNNGEATVSQIGQYVSTAKSALRSAGFTGPVLSVDTFIAVINNPGLCDFADEYVAVNAHAFFDGGIAASGAGDWAAEQIQRVSSACGGKDVLIVESGWPSKGDTNGAAVPSKSNQQAAVQSLGQKIGSSCIAFNAFNDYWKADGPFNAEKYWGILDS

SEQ ID NO: 3 - DNA, 1041 bp, artificial
  source 1..1041: mol_type = genomic DNA
atgaaatctcaacttatctttatggctcttgcctctctggtggcctccgctcctttagaacaccaacaacaacatcacaaacatgaaaagagagctgtggtgacacaaaccgttactgttgcagcaggtcaaaccgctgctgctggctctgcccaggccgttgtcacctcctctgctgcgccagcatcggtcgcttcctctgcagcagcatcggcttcttcctcctcttcctcttataccagtggcgcctctggcgatctctcaagcttcaaagatggtaccatcaaatgttcagagttcccatccggcgacggtgtcgtctccgtcagttggttaggatttggaggatggtcttccatcatgaatctccaaggtgggacttctgaatcttgtgagaacggctactactgctcatacgcatgtgaagccggctactccaagacccagtggccttccaatcagccatccgatggaagatccgtaggtggtttgttgtgtaaggacggtttgctataccgatccaacactgcttttgacaccctctgtgttccaggtaagggtaccgcttccgtagagaacaatgtttccaaaggtatctctatctgcagaactgactaccctggttccgaaaacatgtgtgttcccacctgggtcgatgctggaaactccaacactttgaccgttgtcgatgaagacaactactacgaatggcaaggtctcaagaccagtgcccaatactacgtcaacaacgctggtgtcagcgttgaagacggttgtatttggggtgacgaaagtagtggtgtcggaaactgggctcctctagttttgggtgccggatctacaggtggtttaacttacctatctttgatccccaacccaaacaacaagaaggctcccaacttcaacgtcaagatcgttgctactgatgggtcctccatcaacggtgattgtaaatacgagaacggtatcttcgttggtagttcaactgatggttgtactgtcactgttacctctggtagtgccaaacttgtgttttactaa

SEQ ID NO: 4 - protein, 346 aa, pichia pastoris
MKSQLIFMALASLVASAPLEHQQQHHKHEKRAVVTQTVTVAAGQTAAAGSAQAVVTSSAAPASVASSAAASASSSSSSYTSGASGDLSSFKDGTIKCSEFPSGDGVVSVSWLGFGGWSSIMNLQGGTSESCENGYYCSYACEAGYSKTQWPSNQPSDGRSVGGLLCKDGLLYRSNTAFDTLCVPGKGTASVENNVSKGISICRTDYPGSENMCVPTWVDAGNSNTLTVVDEDNYYEWQGLKTSAQYYVNNAGVSVEDGCIWGDESSGVGNWAPLVLGAGSTGGLTYLSLIPNPNNKKAPNFNVKIVATDGSSINGDCKYENGIFVGSSTDGCTVTVTSGSAKLVFY

SEQ ID NO: 5 - DNA, 936 bp, artificial
  source 1..936: mol_type = genomic DNA
atgatctttaatcttaaaacactggctgcggttgcaatctccatttcacaagtgtctgcagtttcctctctgggttttgctctcggaaacaagaacgttgacggaacttgtaagtacttggccgactacgaggccgacttggatactattagaggcggctctgaagccgttgctattagagcttattccgctgaagactgtaacactttacaatacctcggtcctgctgttgaagagaagggcttcaaattagttctatcagtcagaccactggatgagagctactaccaggcagaaaagaatgcactaagtgaataccttccccaattatctgtttcgactttgcaatttttgtcagttggatccgaagctttgtacagagacgacttgccagcttcagatctggctgataaaattagagatatgaaggagtttttggctggcttgactgacaagaatggggactcctactcttccgtcccagtcggaaccatcgattcatggaacgtccttgtagacgcctccgctgcaccagctattgaagcatctgatgccgtttacgccaacgctttctcatactggcaaggtcaaggtccttccaactctacctattccttctttgacgatatcatgcaagcattgcaagtaatccagaccatcaagggatctactgatatcgatttctgggttggtgagaccggatggcctaccgacggtgacaactttggtgatgctgttccatctattgagaacgctgacaacttttggaaagaagctatctgcggtatcagaggttggggcattaacacattcgttttccaggcatttgacgaagactggaaggaagaggacgacgctgttgaaaaccacttcggtgtttgggacagttccagacagttaaagctggactcattaggttgcgacttttcttcttga

SEQ ID NO: 6 - protein, 311 aa, pichia pastoris
MIFNLKTLAAVAISISQVSAVSSLGFALGNKNVDGTCKYLADYEADLDTIRGGSEAVAIRAYSAEDCNTLQYLGPAVEEKGFKLVLSVRPLDESYYQAEKNALSEYLPQLSVSTLQFLSVGSEALYRDDLPASDLADKIRDMKEFLAGLTDKNGDSYSSVPVGTIDSWNVLVDASAAPAIEASDAVYANAFSYWQGQGPSNSTYSFFDDIMQALQVIQTIKGSTDIDFWVGETGWPTDGDNFGDAVPSIENADNFWKEAICGIRGWGINTFVFQAFDEDWKEEDDAVENHFGVWDSSRQLKLDSLGCDFSS

SEQ ID NO: 7 - DNA, 1845 bp, artificial
  source 1..1845: mol_type = genomic DNA
atgagcaccctgacattgctggctgtgctgttgtcgcttcaaaattcagctcttgctgctcaagctgaaactgcatccctatatcaccaatgtggtggtgcaaactgggagggagcaacccagtgtatttctggtgcctactgtcaatcgcagaacccatactactatcaatgtgttgctacttcttggggttactacactaacacctcaatctcttcgacggccacccttccttcttcttctactactgtctctccaaccagcagtgtggtgcccactggcttggtgtccccattgtatgggcaatgtgggggacagaattggaatggagccacatcttgtgctcagggaagctactgcaagtatatgaacaattattacttccaatgtgttcctgaagctgatggaaaccctgcagaaattagcactttttccgagaatggagagattatcgttactgcaatcgaagctcctacatgggctcaatgtggtggtcatggctactacggcccaactaaatgtcaagtgggaacatcatgccgtgaattaaacgcttggtattatcagtgtatcccagacgatcacaccgatgcctctactaccactttggatcctacttccagttttgtgagtacgacatcattatcgactcttccagcttcttcagaaacgacaattgtaactcctacctcaattgctgctgagcaagtacctctttggggacaatgtggaggaattggttacactggctctacgatttgtgagcagggatcgtgtgtttacttgaacgattggtactatcagtgtctaataagtgatcaaggtacagcatcaactaccagtgcaacgactagtataacttccttcaatgtttcatcgtcgtcagaaacgacggtaatagcccctacctcaatttctactgaggatgtcccactttggggccaatgtggaggaattggatataccggttcgaccacttgtagccagggatcatgcgtttacttaaatgactggtattttcaatgtttaccagaggaggaaacgacttcatcaacttcgtcatcttcctcatcttcctcatcttccacatcttccgcatcttccacatcttccacatcatccacatcctccacatcctccacatcttcctcaacaagtagctcatccattccgacttctacaagctcatcgggagactttgagacaatccccaacggtttctcgggaactggaagaaccacgagatattgggattgttgtaagccaagctgctcatggcctgggaaatccaacagcgtaacaggaccagtgagatcttgtggtgtttctggcaacgtcctggacgccaacgcccaaagtggatgtattggtggtgaagctttcacttgtgatgagcaacaaccttggtccatcaatgacgacctagcctatggttttgccgcagcaagcctagctggtggatctgaggattcctcttgctgcacctgtatgaagctgacattcacctcatcttccattgctggaaagacaatgatcgttcaactgaccaatactggagctgatcttggatcgaatcactttgacattgctcttcctggtggagggcttggaatcttcaccgaaggatgctctagtcaatttggaagcggttaccaatggggtaaccagtatggtggtatctcttcgcttgctgagtgtgatggcctaccatcagaactgcagccaggctgtcagtttagatttggctggtttgagaacgctgataacccttcagtggagtttgaacaggtttcatgtcctccggaaatcacttctatcaccggctgtgctcgtacggacgaataa

SEQ ID NO: 8 - protein, 614 aa, pichia pastoris
MSTLTLLAVLLSLQNSALAAQAETASLYHQCGGANWEGATQCISGAYCQSQNPYYYQCVATSWGYYTNTSISSTATLPSSSTTVSPTSSVVPTGLVSPLYGQCGGQNWNGATSCAQGSYCKYMNNYYFQCVPEADGNPAEISTFSENGEIIVTAIEAPTWAQCGGHGYYGPTKCQVGTSCRELNAWYYQCIPDDHTDASTTTLDPTSSFVSTTSLSTLPASSETTIVTPTSIAAEQVPLWGQCGGIGYTGSTICEQGSCVYLNDWYYQCLISDQGTASTTSATTSITSFNVSSSSETTVIAPTSISTEDVPLWGQCGGIGYTGSTTCSQGSCVYLNDWYFQCLPEEETTSSTSSSSSSSSSSTSSASSTSSTSSTSSTSSTSSSTSSSSIPTSTSSSGDFETIPNGFSGTGRTTRYWDCCKPSCSWPGKSNSVTGPVRSCGVSGNVLDANAQSGCIGGEAFTCDEQQPWSINDDLAYGFAAASLAGGSEDSSCCTCMKLTFTSSSIAGKTMIVQLTNTGADLGSNHFDIALPGGGLGIFTEGCSSQFGSGYQWGNQYGGISSLAECDGLPSELQPGCQFRFGWFENADNPSVEFEQVSCPPEITSITGCARTDE

SEQ ID NO: 9 - DNA, 291 bp, artificial
  source 1..291: mol_type = genomic DNA
atgactaactcagatgtacaacacttaaaacaacaaatacaagatgtgttggtcgagtctggaaagtatgacgaactatctaacttcttgaggtcaaagctataccaagtgggatggactgacgaaattaaccgtctgactcaatccatcgttaccaatgaagctaaacccacatttagtaatgttatcgagaggatcgaaccaaaggcaatggatatagtacctgagcatatcaagacagagatcctggcaaagatagaagagttcttgaaggacgttgttccaaagtaa

SEQ ID NO: 10 - protein, 96 aa, artificial
MTNSDVQHLKQQIQDVLVESGKYDELSNFLRSKLYQVGWTDEINRLTQSIVTNEAKPTFSNVIERIEPKAMDIVPEHIKTEILAKIEEFLKDVVPK

SEQ ID NO: 11 - DNA, 1029 bp, artificial
  source 1..1029: mol_type = genomic DNA
atgacagcattaactgaagagggaagttttaaaggacctgatttgaacgtcgccttgatatgcagagattgcaaagttgatcctcccgaacttattgaacgtttctcagagggtgacgtcatatgtggattatgtggactggtcctgtccgaacacattgttgatatgaggagtgagtggagaaccttcaataacgacgatcagaatggtgacgatccttcaagagttggtgaagctcagaaccctttattggacggagatcaattatcaaccattattgcctataataccgacaatacgcgtatgggacgagaactttccagagctcaaaattccacggttgctgaccgtaaggattcagctttacaagctgctttcgcaaaaatcagtcaactttgcgaaggattccagctgcctaacattgttcagaatggtgctaaagaggtttataagcttgtttacaacgagaggagtttgaagggtaaaagtcaagagtcaattatggcagctgctatcggcttggcatgtcgtaaggctaatgtaccacgttcattcaaagaactttgggcactgactgatgtacccaaaaacgagattggtaaggtctttaagattatccataaactgatccaacaaaagcatgctttggcaggcggactgttaaacgtgcagaacgagtctatagctaccactcaaactaatgctgaggccctgattggaaggttttgttctaatttgggcctttctcgacagattaccaacgctgccgaatacatagctagaaggactaaagaggtaggagtccttgcaggacgttctccagttactgtggctgctacagtaatctacatggccgctagtatattcgatgcttctatttctccagcacaaattgctcagagagctggtgtttcagatggcactattaagacctcttacaaatatctgtacgacaaaagagaagagttagttgaccctcaatggatagagtccggcaaggtcaaactggaaaatatccctaaaaattaa

SEQ ID NO: 12 - protein, 342 aa, pichia pastoris
MTALTEEGSFKGPDLNVALICRDCKVDPPELIERFSEGDVICGLCGLVLSEHIVDMRSEWRTFNNDDQNGDDPSRVGEAQNPLLDGDQLSTIIAYNTDNTRMGRELSRAQNSTVADRKDSALQAAFAKISQLCEGFQLPNIVQNGAKEVYKLVYNERSLKGKSQESIMAAAIGLACRKANVPRSFKELWALTDVPKNEIGKVFKIIHKLIQQKHALAGGLLNVQNESIATTQTNAEALIGRFCSNLGLSRQITNAAEYIARRTKEVGVLAGRSPVTVAATVIYMAASIFDASISPAQIAQRAGVSDGTIKTSYKYLYDKREELVDPQWIESGKVKLENIPKN

SEQ ID NO: 13 - DNA, 1230 bp, artificial
  source 1..1230: mol_type = genomic DNA
atggtatcgctgttacctactgttaacaagtttgaactgccaccactatctgcaatattgaatgaatcacctcttcgtaaccagttgggccatgagagaactcgaagtacaagccggcctggttctccgttaatgtctcatcagttaagtcctgctagcatttcacgaaaagatgttcacacacttccgcctttcggtccgttggatagtaacgttgtggcgatgcaaggcaaacctgacccaacatttggcactccggttttttccagagtgaccaatccttctttccagcatacacctgaatctatatctgtaccgaaaacgctttctgttacgagtctagattcttccgcaaagaagactccacagaatacaaaattatttgcattcatttcccattctccggagacatttcctctacaagaacctaccatagataatgcacaacttgcccgaaggaagagaagaagaacgtcgcccgctgaactattcattcttaaggaagagttttcaaaagggagtactccaaacagagctcgaagaaaggagatttccaggcgagtcaacatgactgataaagctgttcaagtttggtttcaaaatagaaggcaatcgatgcgcaagcataatcaagcaaaacaagaaatacttctagatcctgttatacctcaaccgatttcccagcagttgcattttacaacctcccctttacgttcgaattcttacttcacagattcagataatggtcaagttcacaactctatcccaaattctgatcaaagccagagtccctctcattttcctcctcaaggtacttggctaaacacatctgcagttgtttccaccccaatcaagcaactaatctctaggtcatcaatcactaatgatttcggatcaactatgactttcagactgcaagcaactggaccacgtccaagaaaatcctcatcaccgttcagttctggttctggatctgccaaccgaaacctagtgcatgtgagtgaaagaatggacgctgaatttctgaacaaaccgatcatgaaagttagtcaacaaaacttcgattttaaacgaggtttggataacgccaagacaccgtccaaacaattagtccttcaagacaaatctagaagcgaactcaacaagtcgaactcagcaccaagtatcaaaattagcagagacgaagacgaagaatgtgtcaagcaacttctaagtttacatagctcttga

SEQ ID NO: 14 - protein, 409 aa, pichia pastoris
MVSLLPTVNKFELPPLSAILNESPLRNQLGHERTRSTSRPGSPLMSHQLSPASISRKDVHTLPPFGPLDSNVVAMQGKPDPTFGTPVFSRVTNPSFQHTPESISVPKTLSVTSLDSSAKKTPQNTKLFAFISHSPETFPLQEPTIDNAQLARRKRRRTSPAELFILKEEFSKGSTPNRARRKEISRRVNMTDKAVQVWFQNRRQSMRKHNQAKQEILLDPVIPQPISQQLHFTTSPLRSNSYFTDSDNGQVHNSIPNSDQSQSPSHFPPQGTWLNTSAVVSTPIKQLISRSSITNDFGSTMTFRLQATGPRPRKSSSPFSSGSGSANRNLVHVSERMDAEFLNKPIMKVSQQNFDFKRGLDNAKTPSKQLVLQDKSRSELNKSNSAPSIKISRDEDEECVKQLLSLHSS

SEQ ID NO: 15 - DNA, 2226 bp, artificial
  source 1..2226: mol_type = genomic DNA
atggaaattttaaaagaagaagcgacggaaagcaacggtaaaagaaagctcgaggaggaaagtgatgccttgcaattgtccaaacaagaaggtgagggccatctttccggattacctccctcaggtaaatgggacgataaccaaatcgttaacgggtcggtaattgtccccgtggtagaacctaaacttagatatattacgctcaagactggtttatgttatgatgtgcgcatgaggtatcatgccaaaattttcacgtcctactttgagtacatcgatccacaccctgaagaccctagaaggatatatcgtatttataagatactagcagaaaatgggcttatcacagatccaacgctgtctggaatagatcaaatcggtgactatatgctcaaaatccctgttagagaagccacggcggaggaaattctattggtacattcagaagagcatttgaaatttatagagagtacttcaagcatgtccagagagaggcttctagaggaaacggaaaaaggggattcggtgtacttcaaccatgattctttgctaagtgctaagttatcttgtgggggagccattgaagcgtgtaaggcagtcgtcgaaggaagggttaagaatgccctcgctgtggtcaggcctccagggcatcatgcagagccagactccccaggaggattctgccttttttccaatgtcgccgtagctgccaaaaacattctcaggaactaccctgaatcggtcagaaaaatagtagttctcgattgggatgttcatcatggaaacggtacccaaaaggctttttgggaagaccccagagttctatatatctctctgcatcgttacgagcagggcaaatactaccctgggacaaaagctggaggagctgatcaatgtggagaaaatgaaggtttagggaaaaacatcaacatcccttggcctgttggaggtatgaacgacgctgattacctctatgcctttagaaaagttgtcatgcctgtttgcagggaatacgcacccgacttgctaatcatttcctctgggtttgacgctgctgaaggagatatcattgggggatgtcatatatcgcccgctggttacagtcaaatgacccacatgctaaagtcccttgcacggggaaacgtgtgtgttgttctagaaggtggatataacctggattcgatagcaaactctgcattaagtgttaccaaagtgctcttgggtgaatcacctgaagaacccaaagtcacagtaccaagtgctcatgctattgaagtcatagatgatgtcatcaaaattcaatctcagtattggaaaactctccaacccgcatacacaggaatatgttttacaaacccttcaattatgggtaattactctttactagtaaatccagccactgaaaagaaagttctcagcgatctcgcagttaatccaagactatgcgatgctgttagaaattcccaagctcagtatttgtcgtccaagtttggtttcattaatctgccagttgtttcaggcaaaggattgacttctccatctctggataaccaggttctgtcaacaaaggacatcttccaagccaataccataataatagtaatacacgatccatccgatgtatgggccagacaagacccgaggtctggactgctggatctctccgggtctatgatagtcgacacctcttctaaattcgttgaatgggctgtgaacttgaaatatggagttatagatataaatgttccattgacattgacaggcaaggatgatgaaacatacaacaacgttacagcttctcaggagctactcctttatatttgggacaattacattcagtactttccagttacaaaaattgcacttgttggattcggtgatgcttacaatggagtcatacacctttgtggtcatcgagaagtccgcagcatagtgaaagcttctatcaacttcctggatagaactccgttacgtgctattgtttccagcatagatgaatctgtcactgactggttttataaaaactcactagttttcactagtactaggcatccttgttggggagaacagggaaccagtgaaatgaagagacctcgtaaaaagtatggtagagtgctgaaggctgacatagatggactgccaaatattgttgatgaaagatttgaggaaactaccgactttattttagactccatcgaagaatacgaagatgagagttctaactaa

SEQ ID NO: 16 - protein, 741 aa, pichia pastoris
MEILKEEATESNGKRKLEEESDALQLSKQEGEGHLSGLPPSGKWDDNQIVNGSVIVPVVEPKLRYITLKTGLCYDVRMRYHAKIFTSYFEYIDPHPEDPRRIYRIYKILAENGLITDPTLSGIDQIGDYMLKIPVREATAEEILLVHSEEHLKFIESTSSMSRERLLEETEKGDSVYFNHDSLLSAKLSCGGAIEACKAVVEGRVKNALAVVRPPGHHAEPDSPGGFCLFSNVAVAAKNILRNYPESVRKIVVLDWDVHHGNGTQKAFWEDPRVLYISLHRYEQGKYYPGTKAGGADQCGENEGLGKNINIPWPVGGMNDADYLYAFRKVVMPVCREYAPDLLIISSGFDAAEGDIIGGCHISPAGYSQMTHMLKSLARGNVCVVLEGGYNLDSIANSALSVTKVLLGESPEEPKVTVPSAHAIEVIDDVIKIQSQYWKTLQPAYTGICFTNPSIMGNYSLLVNPATEKKVLSDLAVNPRLCDAVRNSQAQYLSSKFGFINLPVVSGKGLTSPSLDNQVLSTKDIFQANTIIIVIHDPSDVWARQDPRSGLLDLSGSMIVDTSSKFVEWAVNLKYGVIDINVPLTLTGKDDETYNNVTASQELLLYIWDNYIQYFPVTKIALVGFGDAYNGVIHLCGHREVRSIVKASINFLDRTPLRAIVSSIDESVTDWFYKNSLVFTSTRHPCWGEQGTSEMKRPRKKYGRVLKADIDGLPNIVDERFEETTDFILDSIEEYEDESSN

SEQ ID NO: 17 - DNA, 1758 bp, artificial
  source 1..1758: mol_type = genomic DNA
gacgcccacaaaagtgaagtagcacaccgttttaaagatttaggtgaagaaaactttaaggctttagttctgattgcattcgctcaatatttgcaacagtgtcccttcgaagatcacgtgaaactagtcaatgaggtgaccgaattcgctaagacttgtgttgccgacgagagtgctgaaaactgtgataagtccttacatacgctattcggagacaaattgtgcacagtggcaactttgagagagacctacggagaaatggcagactgttgtgccaaacaggaaccagagagaaatgaatgtttcttgcaacataaggatgacaaccctaaccttcctagacttgttaggcctgaagtggatgttatgtgcacagcttttcatgataatgaagagaccttcttgaaaaaatacttgtacgaaatcgccagacgtcatccatacttctatgctccagagttattatttttcgctaaacgttacaaggcagctttcaccgagtgttgtcaagcagctgataaggctgcatgtttactaccaaagttggacgagctacgtgatgaaggtaaggcatcatccgcaaagcagaggctaaaatgtgcctctctgcagaagttcggcgaaagggcttttaaagcatgggccgttgccagactttcacagagattcccaaaagctgaatttgcagaggtttccaagctggttactgatcttactaaagtgcatactgaatgttgtcatggtgatctattagaatgtgctgacgaccgtgctgacttggccaaatatatatgcgaaaaccaggactctatttcatccaagttgaaggaatgctgtgagaaacctcttttagaaaagtcccactgcatcgctgaagttgaaaatgacgaaatgccagcagacctaccatctctggcagctgatttcgttgaatcaaaggacgtctgtaaaaactacgctgaagcaaaggatgtttttctgggcatgtttttgtatgaatatgctagaaggcatccagattatagtgttgttcttcttttgaggttggctaagacctacgagacaacactggagaagtgttgcgctgctgccgatccacacgagtgttacgccaaagtgtttgacgaatttaagcctttagttgaggagccccaaaatcttattaagcaaaattgtgaactattcgaacagcttggtgaatataagtttcaaaacgcactactggtgaggtatacaaaaaaggtcccacaagtttccacgccaacattggtagaagtctctagaaatttgggaaaggtcggtagtaagtgttgcaaacacccagaagctaaacgaatgccatgcgcagaagattacctgtctgttgtgttgaaccagctttgcgttcttcacgaaaaaactcctgtgtctgatagggttacaaaatgttgtactgagagtttggtgaacagaagaccttgtttttctgctctagaggttgacgagacatacgtccctaaagagttcaacgctgagactttcactttccacgctgacatttgcaccctgtcagagaaggaacgacaaattaagaaacaaacggccttagttgaattagttaagcataagccaaaagcaacgaaggagcagcttaaagctgttatggatgactttgcagcctttgttgagaagtgttgtaaagcagatgataaagagacatgctttgctgaagagggaaaaaagttagttgccgcttctcaagctgcccttggtctataa

SEQ ID NO: 18 - DNA, 1758 bp, artificial
  source 1..1758: mol_type = genomic DNA
gatgcacataaatctgaagtagctcatcgtttcaaggacttgggtgaagaaaacttcaaggctctagttttaatcgctttcgctcaatatttacagcaatgtccctttgaggatcacgtaaagttggtcaacgaggttacagaatttgctaaaacctgtgtcgccgatgaatctgctgaaaactgcgataaatctcttcatacccttttcggagacaaattgtgtacggtcgccactttgagagaaacttacggcgaaatggcagattgctgtgctaaacaagaaccagagagaaatgaatgtttcttgcaacataaggatgataacccaaatttacctagattagtgagacccgaagtagacgttatgtgtactgcatttcatgataacgaggagacttttctgaaaaagtatttgtatgaaattgcccgtagacacccatacttctatgcaccagaacttctgtttttcgccaaaagatataaagctgcattcaccgaatgttgccaagcagctgataaagctgcatgcttgcttcccaaattggacgagttaagagatgaaggtaaagcctccagtgctaaacaaagattgaaatgcgcttccctacagaagttcggagagagggcttttaaggcttgggctgtagcaagactttcccagagattccctaaagctgagttcgcagaggtcagtaagcttgttactgacctgactaaagttcatacggaatgctgtcatggtgacctgttagagtgtgctgatgatagagcagacttggccaagtatatctgtgaaaaccaagactcaatctcctccaagttgaaagaatgttgtgaaaagccacttttggagaaatcccactgtattgccgaagtggaaaacgacgaaatgcccgctgatcttccctctttggctgctgacttcgttgagtccaaggatgtttgcaagaattacgctgaagctaaagacgtattcttaggtatgtttctgtacgagtacgcacgtaggcatccagactactctgttgttcttctgctgcgacttgccaagacttatgaaactacattggaaaaatgctgcgccgctgcagacccacacgaatgctatgcaaaagtctttgacgagtttaagcccttggtcgaggagccacaaaaccttatcaaacagaactgtgaattatttgaacaacttggagaatataagttccaaaatgccttgctggtgagatacactaagaaagttccacaggtatccacacctactctagttgaggttagtagaaacttgggtaaagttggttctaaatgttgtaagcaccctgaagctaaacgtatgccttgtgctgaagattacttgtctgtggtgttaaatcagctgtgtgttttgcatgaaaagacgccagtttctgacagagtgacaaaatgttgcactgagagtctagtgaatagaagaccttgcttcagtgcactagaggtagatgagacctatgttcctaaagaatttaatgcagaaacattcaccttccatgcagatatctgcaccttgagtgagaaagagagacaaatcaagaaacaaacggctttggttgaattagttaagcacaaacccaaggccactaaagagcaacttaaagctgtaatggacgattttgctgccttcgtagaaaagtgttgtaaggccgatgataaagaaacgtgttttgctgaggagggaaagaaattggtcgctgcttcacaagcagctctgggattataa

SEQ ID NO: 19 - DNA, 1755 bp, artificial
  source 1..1755: mol_type = genomic DNA
gaagcccaccaatccgagatagcccatagatttaatgatttaggagaagaacatttccgtggtttagtattagttgccttttctcaatacctgcaacagtgcccattcgaagatcatgttaagttggttaatgaagttaccgagtttgcaaaaggatgtgttgctgaccagtcagctgcaaactgtgagaagtcattacatgaattgttgggtgataaactatgtaccgtagcaagtctacgtgataagtacggtgaaatggcagattgttgtgaaaaaaaagaacctgaacgtaacgaatgctttctacaacataaagacgacaatcctggattcggccaattggttaccccagaagcagacgcaatgtgtaccgcctttcatgagaacgagcagcgttttcttggcaagtatctgtatgaaatcgcacgaagacatccctacttctacgctcctgaactactgtactatgctgaagagtacaaaggtgtgttcaccgaatgttgtgaagctgcagataaagcagcttgtttaactccaaaggtggatgcacttagagagaaggttttggcatcctctgccaaagaaaggttgaaatgcgcctcactgcagaaattcggtgagagagctttcaaggcctggtctgttgctagactatctcaaaagttccctaaggctgaatttgcagagatttcaaagctagttaccgatctggcaaagatacataaagagtgttgtcacggagatttgttagaatgcgctgacgatcgtgctgatttagctaagtatatctgcgagaaccaggactccatatccacaaagttgaaagaatgttgtggtaaaccagtcttagagaagtcccactgcatttccgaagtggaaagagacgaactacccgccgacttacctcctttagcagttgatttcgtcgaagacaaggaagtttgtaagaattaccaagaggctaaagatgttttcctgggtaccttcttgtatgaatatagtagaagacaccctgagtactctgtctctctattactgcgtctggctaaagaatacgaggctactctagagaagtgttgcgccacagatgaccctccagcttgttatgcacatgtttttgacgaatttaagcccctggttgaggaaccacataacttagtgaagaccaactgcgaattgttcgaaaagttgggagaatacggattccagaatgctcttcttgtgagatacacgaaaaaggtgccacaagtctctaccccaactttggtcgaggtttctagatcattgggaaaagttggatccaaatgttgtactcaccctgaagccgagagactttcatgtgctgaggattatttatccgtagttcttaaccgtctatgtgttcttcacgagaagactccagtgtccgagagggttaccaagtgttgtactgagtcacttgtaaatagaagaccctgtttctccgccctgcaagttgatgagacatatgtccccaaggaattcagtgctgaaaccttcacattccatgccgacttatgcactctgcctgaggccgaaaagcaaattaaaaagcaatctgcacttgtggaactgttgaaacataagcctaaagcaaccgaagaacaattgaaaactgtaatgggcgattttggatcttttgtggacaagtgttgcgcagccgaggataaagaggcatgtttcgccgaggaaggacctaaattggtagctgctgcccaagccgcactagcttaa

SEQ ID NO: 20 - DNA, 1755 bp, artificial
  source 1..1755: mol_type = genomic DNA
gaagcttataaatcagagatagcacacagatataacgacttgggtgaagagcactttagaggattggtgctggtggcattctcccaatacttgcaacagtgcccattcgaagatcatgtcaagctggctaaggaagtgacggaatttgccaaagcttgtgctgctgaagaatcaggtgcaaactgtgacaaatcactacatactttgttcggcgacaagttgtgtaccgtggcttctttaagggacaagtatggcgatatggcagattgttgtgaaaaacaagagccagacagaaacgagtgtttcctagctcacaaggatgataacccaggatttcctcctctagttgcaccagaacctgatgcattgtgtgcagctttccaggacaacgaacagctttttcttggaaagtacctatatgagatagccaggcgtcatccatacttctatgcaccagagcttttgtactacgcccaacaatacaagggagtattcgccgagtgttgccaagccgctgataaagctgcttgcttaggtccaaaaattgaagccttgagagaaaaggttttgttgagttcagcaaaagaaagatttaagtgcgcttcactgcaaaagtttggtgatagggcctttaaggcctggagtgttgcaagattgagtcagcgtttcccaaaggctgattttgcagaaatttccaaggtcgtgaccgatttaaccaaagtgcataaagaatgctgtcacggtgacctgttggaatgtgcagatgacagagctgatctggccaaatacatgtgcgaaaaccaggactctatttcaactaaattgaaagagtgttgcgacaagcctgttctagagaagtcccaatgtttagctgaagttgagagagacgagttaccaggtgacttgccctccctggccgcagattttgtggaagacaaagaggtgtgtaagaattatcaggaagcaaaagacgttttcctgggtacttttttatacgagtacgctcgaagacaccctgagtattctgtttctctgcttcttagattggcaaaggaatacgaagccactctggagaaatgctgtgctactgatgacccccctacttgttacgctaaggtattggacgaattcaagcctttggttgatgagccacaaaatctggtgaaaaccaattgcgaactgtttgagaagttgggtgaatatggtttccagaacgctcttctggttagatatacaaaaaaagcacctcaggtctctacaccaactttagtcgaggtcagtaggaagttgggtaaagttggtacgaagtgctgcaaaaagccagagtccgaaagaatgtcttgtgctgaagactttttgtcagtggtccttaaccgactgtgcgttttacatgaaaagaccccagtttctgaacgtgttactaagtgttgttcagaatctctggtaaatagacgtccatgcttttcaggactggaagttgatgaaacctacgtcccaaaagaattcaacgctgaaacatttacctttcatgctgatttatgtacccttcctgaagctgaaaagcaagtcaagaaacagaccgctctagtcgaattgttgaaacacaaacccaaggcaacagatgagcagttgaagactgttatgggtgatttcggtgcattcgttgaaaaatgctgcgcagctgagaacaaagagggttgcttttccgaggagggtcctaagcttgttgctgctgctcaagcagctctggtctaa

SEQ ID NO: 21 - DNA, 1752 bp, artificial
  source 1..1752: mol_type = genomic DNA
gatacacataaaagtgaaattgcccatagattcaaagacctaggtgaggaacacttcaaaggattggttctgattgcctttagtcagtaccttcaacagtgtcccttcgatgaacacgtgaagttagttaatgaacttaccgagtttgctaaaacttgcgttgccgatgaatctcatgctggttgtgaaaagtcattgcatactttgttcggtgatgagctatgtaaagtcgccagtctgagagagacttatggagatatggctgactgctgcgaaaaacaagagcctgagagaaacgagtgtttcttgtcacataaggatgactctccagacctacctaaattgaagccagatcccaataccctttgtgacgagttcaaagccgacgaaaaaaagttctggggtaagtatttgtatgagattgcccgtagacatccatacttctacgctcccgagttgctgtattacgctaataagtataacggtgtcttccaggaatgttgtcaagcagaggataagggtgcttgtttgcttccaaagattgaaactatgagagaaaaggttttggcatcttctgccagacagagattgaggtgcgcctccatacagaagttcggagaaagagccttgaaagcctggtcagtggccaggctaagtcagaaattccctaaggctgagttcgtggaagttactaagctggttaccgatctgactaaagtacacaaggaatgttgtcatggagatttgcttgaatgtgctgatgatcgagcagacttggctaagtacatttgtgacaatcaggatacaatttcttcaaagcttaaagagtgctgtgataaacctttgctggagaagtcacattgtatcgcagaagtcgaaaaggatgctatcccagaaaacttgcctccattaaccgcagacttcgctgaagataaggatgtttgcaaaaattaccaggaagcaaaagacgcttttttgggctcttttctttatgaatattccaggagacacccagaatatgctgtatctgtgttgttgcgtcttgcaaaagaatatgaagccaccctagaagaatgttgtgccaaggacgatccacacgcttgttattcaaccgttttcgataaattgaagcaccttgtcgatgaaccacagaacttgattaagcaaaattgtgatcaatttgaaaaactgggtgagtatggttttcagaacgccctaattgttcgttatactagaaaggttccacaagtatcaacacccactctagtcgaggtaagtagaagtttgggcaaagtcggaacaagatgctgcactaagccagaatccgaaagaatgccatgtaccgaggattacctatcattgattttaaatagactttgtgttctgcacgagaagacaccagtttctgaaaaagtcacgaaatgttgtaccgagagtttggttaacaggagaccctgtttttcagccttaacaccagatgaaacctacgtacctaaggcttttgacgaaaagctgtttacctttcatgcagatatctgcactttgcctgacaccgaaaaacagattaaaaaacagactgcacttgtggaacttttgaaacataagccaaaggctactgaggaacagttaaagacggtgatggagaacttcgtagcctttgttgacaaatgttgcgccgctgacgacaaagaggcatgctttgctgttgaaggtccaaagttggttgtttcaacacagactgctttggcttaa

SEQ ID NO: 22 - DNA, 1752 bp, artificial
  source 1..1752: mol_type = genomic DNA
gatactcataaaagtgaaattgctcatcgattcaatgaccttggcgagaaacatttcaagggtttggtgctggtggctttctctcagtatcttcaacagtgtcctttcgaagaccatgtaaagttggtaaacgaagtaactgaattcgccaaaaaatgtgcagctgacgaatccgctgaaaattgcgataagagtcttcacactttgtttggtgataagctgtgtaccgtagccactttaagagctacctacggagagttggcagattgttgcgagaagcaagagccagaaagaaatgagtgttttttgactcataaggacgatcatcccaatttaccaaagcttaagcctgaacctgacgctcaatgcgcagctttccaagaggatccagacaagttcctgggtaagtacctatacgaggttgctagaagacatccatatttctacggacctgagctactgtttcatgctgaagagtataaagctgacttcactgaatgctgtcccgctgatgataaacttgcctgtttgataccaaaactggacgctttgaaggaacgtattcttttgtcctctgctaaagagcgtttaaagtgctcctcttttcagaactttggtgaaagagccgttaaagcatggtcagtcgctagattgtctcaaaagtttcctaaagctgacttcgcagaagtttctaaaattgttacggacttgactaaggttcataaggaatgttgtcatggtgatttgctggaatgtgcagatgatagagccgacctggcaaagtatatttgcgaacaccaggattccatttccggtaagctaaaagcatgttgtgacaagcccctgcttcaaaagtcccactgcattgctgaagttaaagaggatgatttgccatctgatttgcccgctttagccgctgatttcgccgaagacaaagaaatctgcaaacactacaaggatgcaaaagatgttttcctgggaacctttttgtacgaatattcacgtcgacatccagattactccgttagtctgttactacgtatcgccaagacttatgaagctactttggaaaaatgttgtgctgaggccgatcctccagcttgttatcgtaccgtttttgatcaatttactcctcttgtcgaggaacccaaatctttggtgaaaaagaattgcgatttgtttgaggaagttggagagtatgatttccaaaacgctttaatagttagatacacgaagaaagctccccaggtctctactcctaccttggtagagattggaaggactctgggcaaggttggatctagatgctgcaaacttcctgaatctgaacgtctaccttgttccgaaaatcacctggctttggctttaaatcgtttatgcgttctgcatgaaaagacccctgtgtccgagaagattaccaagtgttgcactgattcactagccgagagaaggccttgcttctcagctttggagttggacgaaggttatgtacccaaagaattcaaagctgagactttcacttttcatgccgacatttgtactcttcctgaagatgagaagcaaattaagaaacaatcagccttggctgaattggttaaacacaaacctaaggcaactaaggaacagttgaagacagtgttaggtaactttagtgcatttgtggctaagtgttgtggcagagaggataaggaagcctgtttcgctgaggagggacccaagttggttgcttcatcccaacttgccttagcttaa

SEQ ID NO: 23 - DNA, 20 bp, artificial
  source 1..20: mol_type = other DNA
gctcacgctttctttgacgg

SEQ ID NO: 24 - DNA, 20 bp, artificial
  source 1..20: mol_type = other DNA
ggtgattgtaaatacgagaa

SEQ ID NO: 25 - DNA, 20 bp, artificial
  source 1..20: mol_type = other DNA
attctgtggagtcttctttg

SEQ ID NO: 26 - DNA, 20 bp, artificial
  source 1..20: mol_type = other DNA
aatggagtcatacacctttg

SEQ ID NO: 27 - DNA, 4128 bp, artificial
  source 1..4128: mol_type = genomic DNA
atggacaagaagtactccattgggctcgatatcggcacaaacagcgtcggctgggccgtcattacggacgagtacaaggtgccgagcaaaaaattcaaagttctgggcaataccgatcgccacagcataaagaagaacctcattggcgccctcctgttcgactccggggagacggccgaagccacgcggctcaaaagaacagcacggcgcagatatacccgcagaaagaatcggatctgctacctgcaggagatctttagtaatgagatggctaaggtggatgactctttcttccataggctggaggagtcctttttggtggaggaggataaaaagcacgagcgccacccaatctttggcaatatcgtggacgaggtggcgtaccatgaaaagtacccaaccatatatcatctgaggaagaagcttgtagacagtactgataaggctgacttgcggttgatctatctcgcgctggcgcatatgatcaaatttcggggacacttcctcatcgagggggacctgaacccagacaacagcgatgtcgacaaactctttatccaactggttcagacttacaatcagcttttcgaagagaacccgatcaacgcatccggagttgacgccaaagcaatcctgagcgctaggctgtccaaatcccggcggctcgaaaacctcatcgcacagctccctggggagaagaagaacggcctgtttggtaatcttatcgccctgtcactcgggctgacccccaactttaaatctaacttcgacctggccgaagatgccaagcttcaactgagcaaagacacctacgatgatgatctcgacaatctgctggcccagatcggcgaccagtacgcagacctttttttggcggcaaagaacctgtcagacgccattctgctgagtgatattctgcgagtgaacacggagatcaccaaagctccgctgagcgctagtatgatcaagcgctatgatgagcaccaccaagacttgactttgctgaaggcccttgtcagacagcaactgcctgagaagtacaaggaaattttcttcgatcagtctaaaaatggctacgccggatacattgacggcggagcaagccaggaggaattttacaaatttattaagcccatcttggaaaaaatggacggcaccgaggagctgctggtaaagcttaacagagaagatctgttgcgcaaacagcgcactttcgacaatggaagcatcccccaccagattcacctgggcgaactgcacgctatcctcaggcggcaagaggatttctacccctttttgaaagataacagggaaaagattgagaaaatcctcacatttcggataccctactatgtaggccccctcgcccggggaaattccagattcgcgtggatgactcgcaaatcagaagagaccatcactccctggaacttcgaggaagtcgtggataagggggcctctgcccagtccttcatcgaaaggatgactaactttgataaaaatctgcctaacgaaaaggtgcttcctaaacactctctgctgtacgagtacttcacagtttataacgagctcaccaaggtcaaatacgtcacagaagggatgagaaagccagcattcctgtctggagagcagaagaaagctatcgtggacctcctcttcaagacgaaccggaaagttaccgtgaaacagctcaaagaagactatttcaaaaagattgaatgtttcgactctgttgaaatcagcggagtggaggatcgcttcaacgcatccctgggaacgtatcacgatctcctgaaaatcattaaagacaaggacttcctggacaatgaggagaacgaggacattcttgaggacattgtcctcacccttacgttgtttgaagatagggagatgattgaagaacgcttgaaaacttacgctcatctcttcgacgacaaagtcatgaaacagctcaagaggcgccgatatacaggatgggggcggctgtcaagaaaactgatcaatgggatccgagacaagcagagtggaaagacaatcctggattttcttaagtccgatggatttgccaaccggaacttcatgcagttgatccatgatgactctctcacctttaaggaggacatccagaaagcacaagtttctggccagggggacagtcttcacgagcacatcgctaatcttgcaggtagcccagctatcaaaaagggaatactgcagaccgttaaggtcgtggatgaactcgtcaaagtaatgggaaggcataagcccgagaatatcgttatcgagatggcccgagagaaccaaactacccagaagggacagaagaacagtagggaaaggatgaagaggattgaagagggtataaaagaactggggtcccaaatccttaaggaacacccagttgaaaacacccagcttcagaatgagaagctctacctgtactacctgcagaacggcagggacatgtacgtggatcaggaactggacatcaatcggctctccgactacgacgtggatcatatcgtgccccagtcttttctcaaagatgattctattgataataaagtgttgacaagatccgataaaaatagagggaagagtgataacgtcccctcagaagaagttgtcaagaaaatgaaaaattattggcggcagctgctgaacgccaaactgatcacacaacggaagttcgataatctgactaaggctgaacgaggtggcctgtctgagttggataaagccggcttcatcaaaaggcagcttgttgagacacgccagatcaccaagcacgtggcccaaattctcgattcacgcatgaacaccaagtacgatgaaaatgacaaactgattcgagaggtgaaagttattactctgaagtctaagctggtctcagatttcagaaaggactttcagttttataaggtgagagagatcaacaattaccaccatgcgcatgatgcctacctgaatgcagtggtaggcactgcacttatcaaaaaatatcccaagcttgaatctgaatttgtttacggagactataaagtgtacgatgttaggaaaatgatcgcaaagtctgagcaggaaataggcaaggccaccgctaagtacttcttttacagcaatattatgaattttttcaagaccgagattacactggccaatggagagattcggaagcgaccacttatcgaaacaaacggagaaacaggagaaatcgtgtgggacaagggtagggatttcgcgacagtccggaaggtcctgtccatgccgcaggtgaacatcgttaaaaagaccgaagtacagaccggaggcttctccaaggaaagtatcctcccgaaaaggaacagcgacaagctgatcgcacgcaaaaaagattgggaccccaagaaatacggcggattcgattctcctacagtcgcttacagtgtactggttgtggccaaagtggagaaagggaagtctaaaaaactcaaaagcgtcaaggaactgctgggcatcacaatcatggagcgatcaagcttcgaaaaaaaccccatcgactttctcgaggcgaaaggatataaagaggtcaaaaaagacctcatcattaagcttcccaagtactctctctttgagcttgaaaacggccggaaacgaatgctcgctagtgcgggcgagctgcagaaaggtaacgagctggcactgccctctaaatacgttaatttcttgtatctggccagccactatgaaaagctcaaagggtctcccgaagataatgagcagaagcagctgttcgtggaacaacacaaacactaccttgatgagatcatcgagcaaataagcgaattctccaaaagagtgatcctcgccgacgctaacctcgataaggtgctttctgcttacaataagcacagggataagcccatcagggagcaggcagaaaacattatccacttgtttactctgaccaacttgggcgcgcctgcagccttcaagtacttcgacaccaccatagacagaaagcggtacacctctacaaaggaggtcctggacgccacactgattcatcagtcaattacggggctctatgaaacaagaatcgacctctctcagctcggtggagacccaaagaagaaaagaaaagtttaa

SEQ ID NO: 28 - DNA, 4128 bp, artificial
  source 1..4128: mol_type = genomic DNA
atggacaagaagtactccatcggtctggacatcggaactaactctgttggttgggctgttatcaccgacgagtacaaggttccatccaagaagttcaaggtcctgggtaacactgacagacactccatcaagaagaacttgatcggagccttgttgttcgactctggtgaaactgctgaggccaccagattgaagagaactgccagaagaagatacaccagacgtaagaacagaatctgctacctgcaagagattttctccaacgagatggccaaggtcgacgactcatttttccacagattggaagagtccttcctggtcgaagaggataagaagcacgagagacacccaatcttcggtaacatcgttgacgaggttgcttaccacgagaagtacccaactatctaccacctgagaaagaagttggttgactccactgacaaggccgacttgagattgatctacttggctttggcccacatgattaagttcagaggtcacttcttgatcgagggtgacttgaacccagacaactctgacgttgacaagctgttcatccagttggtccagacctacaaccagctgttcgaagagaaccctattaacgcttctggtgttgacgctaaggctatcttgtctgccagattgtccaagtccagaagattggagaacctgatcgctcaattgccaggtgagaagaagaacggtttgttcggtaacttgattgccctgtccttgggtttgaccccaaacttcaagtccaacttcgatttggctgaggacgccaagttgcagttgtctaaggatacttacgacgacgacctggacaacttgttggctcaaattggtgaccagtacgccgacttgtttttggctgctaagaacttgtccgacgccatcttgttgtccgacatcttgagagttaacaccgagatcactaaggctccattgtccgcttccatgatcaagagatacgacgaacaccaccaggacttgactttgttgaaggccttggttagacagcagctgcctgagaagtacaaagaaatcttcttcgatcagtccaagaacggctacgctggttacattgatggtggtgcttctcaagaagagttctacaagttcatcaagcccatcttggagaagatggacggtactgaagagttgctggtcaagttgaacagagaggacttgctgagaaagcagagaaccttcgacaacggttccattccacaccagattcacttgggtgagttgcacgctatcttgcgtagacaagaggacttctacccattcctgaaggacaacagagagaagatcgaaaagatcctgaccttcagaatcccctactacgttggtccattggctagaggtaactctagattcgcttggatgaccagaaagtccgaagagactatcaccccatggaacttcgaagaggttgttgacaagggtgcttccgctcaatccttcatcgagagaatgactaacttcgacaagaacctgccaaacgagaaggtcttgccaaagcactctttgctgtacgagtacttcaccgtctacaacgagctgactaaggtcaagtacgttaccgagggtatgagaaagccagctttcttgtctggtgagcaaaagaaggctatcgtcgacttgctgttcaagaccaacagaaaggttaccgtcaagcagctgaaagaggactacttcaagaaaatcgagtgcttcgactccgtcgagatttccggtgttgaggatagattcaacgcctccttgggaacctaccacgacttgttgaagatcatcaaggacaaggatttcttggacaacgaggaaaacgaggacattttggaggacatcgtcttgaccttgactctgttcgaggacagagagatgattgaggaaagacttaagacttacgcccacctgttcgacgacaaggttatgaagcaactgaagaggcgtagatacaccggttggggtagattgtctagaaagctgatcaacggtatcagagacaagcagtccggtaagactatcctggactttttgaagtccgacggtttcgccaaccgtaacttcatgcaattgatccacgacgactccctgactttcaaagaggacattcagaaggctcaggtttccggtcaaggtgattccttgcatgagcacattgctaacttggctggttccccagctatcaagaagggtatcttgcagaccgttaaggttgtcgacgagttggttaaggttatgggtagacacaagcccgagaacatcgttatcgaaatggctagagagaaccagactacccagaagggtcaaaagaactccagagaaagaatgaagaggatcgaagagggtatcaaagagctgggttcccagattttgaaagagcacccagttgagaacacccagctgcagaacgaaaagctgtacttgtactacttgcagaacggtagagacatgtacgtcgaccaagagctggacattaacagactgtctgactacgacgttgaccacatcgttccacagtcttttctgaaggacgactccatcgacaacaaggtcttgactagatccgataagaacaggggtaagtccgacaacgttccttctgaagaggtcgtcaagaagatgaagaactactggcgtcagttgctgaacgccaagctgattactcagaggaagttcgacaacttgactaaggctgagagaggtggtttgtccgaattggataaggccggtttcatcaagagacagctggtcgagactagacagatcacaaagcacgttgcccaaatcttggactccagaatgaacactaagtacgacgagaacgacaagttgatccgtgaggttaaggtcatcaccctgaagtccaagttggtgtccgatttcagaaaggacttccaattctacaaggtccgtgagatcaacaactaccaccatgctcacgacgcttacttgaacgctgttgttggtactgccctgatcaaaaagtaccctaagctggaatccgagttcgtctacggtgactacaaggtttacgacgtcagaaagatgatcgccaagtccgaacaagagatcggtaaggctactgccaagtactttttctactccaacatcatgaactttttcaagactgagatcaccctggccaacggtgagatcagaaaaagaccactgatcgagactaacggtgaaaccggtgaaatcgtttgggacaagggtagagacttcgccaccgttagaaaggttttgtccatgccacaggtcaacatcgtcaaaaagactgaggttcagaccggtggtttctccaaagagtccatcttgcctaagagaaactccgacaagctgatcgccagaaagaaggattgggacccaaagaagtacggcggtttcgattctccaactgttgcctactccgttttggttgttgctaaggtcgaaaagggcaagtctaagaagctgaagtccgtcaaagaactgctgggtatcactatcatggaaaggtccagctttgagaagaacccaatcgactttttggaggccaagggttacaaagaggtgaagaaggacctgattatcaagctgccaaagtactccctgttcgagttggaaaacggtagaaagagaatgttggcttccgccggtgaattgcaaaagggtaacgaattggctctgccatccaagtacgtcaactttctgtacttggcctctcactacgagaagttgaagggttctccagaggacaacgaacagaagcagttgttcgttgagcagcacaagcactacttggacgagatcattgagcagatttccgagttctccaagcgtgttattttggctgatgccaacctggataaggtcttgtccgcctacaacaagcacagagataagccaattagagagcaggctgagaacatcatccacttgttcactttgactaacctgggtgccccagctgcttttaagtacttcgacactaccatcgacagaaagagatacacctccaccaaagaggttttggacgctactttgatccaccagtccatcactggtctgtacgaaaccagaattgacttgtcccagcttggtggtgaccctaagaagaagagaaaggtctaa

SEQ ID NO: 29 - protein, 1375 aa, Homo sapiens
MDKKYSIGLDIGTNSVGWAVITDEYKVPSKKFKVLGNTDRHSIKKNLIGALLFDSGETAEATRLKRTARRRYTRRKNRICYLQEIFSNEMAKVDDSFFHRLEESFLVEEDKKHERHPIFGNIVDEVAYHEKYPTIYHLRKKLVDSTDKADLRLIYLALAHMIKFRGHFLIEGDLNPDNSDVDKLFIQLVQTYNQLFEENPINASGVDAKAILSARLSKSRRLENLIAQLPGEKKNGLFGNLIALSLGLTPNFKSNFDLAEDAKLQLSKDTYDDDLDNLLAQIGDQYADLFLAAKNLSDAILLSDILRVNTEITKAPLSASMIKRYDEHHQDLTLLKALVRQQLPEKYKEIFFDQSKNGYAGYIDGGASQEEFYKFIKPILEKMDGTEELLVKLNREDLLRKQRTFDNGSIPHQIHLGELHAILRRQEDFYPFLKDNREKIEKILTFRIPYYVGPLARGNSRFAWMTRKSEETITPWNFEEVVDKGASAQSFIERMTNFDKNLPNEKVLPKHSLLYEYFTVYNELTKVKYVTEGMRKPAFLSGEQKKAIVDLLFKTNRKVTVKQLKEDYFKKIECFDSVEISGVEDRFNASLGTYHDLLKIIKDKDFLDNEENEDILEDIVLTLTLFEDREMIEERLKTYAHLFDDKVMKQLKRRRYTGWGRLSRKLINGIRDKQSGKTILDFLKSDGFANRNFMQLIHDDSLTFKEDIQKAQVSGQGDSLHEHIANLAGSPAIKKGILQTVKVVDELVKVMGRHKPENIVIEMARENQTTQKGQKNSRERMKRIEEGIKELGSQILKEHPVENTQLQNEKLYLYYLQNGRDMYVDQELDINRLSDYDVDHIVPQSFLKDDSIDNKVLTRSDKNRGKSDNVPSEEVVKKMKNYWRQLLNAKLITQRKFDNLTKAERGGLSELDKAGFIKRQLVETRQITKHVAQILDSRMNTKYDENDKLIREVKVITLKSKLVSDFRKDFQFYKVREINNYHHAHDAYLNAVVGTALIKKYPKLESEFVYGDYKVYDVRKMIAKSEQEIGKATAKYFFYSNIMNFFKTEITLANGEIRKRPLIETNGETGEIVWDKGRDFATVRKVLSMPQVNIVKKTEVQTGGFSKESILPKRNSDKLIARKKDWDPKKYGGFDSPTVAYSVLVVAKVEKGKSKKLKSVKELLGITIMERSSFEKNPIDFLEAKGYKEVKKDLIIKLPKYSLFELENGRKRMLASAGELQKGNELALPSKYVNFLYLASHYEKLKGSPEDNEQKQLFVEQHKHYLDEIIEQISEFSKRVILADANLDKVLSAYNKHRDKPIREQAENIIHLFTLTNLGAPAAFKYFDTTIDRKRYTSTKEVLDATLIHQSITGLYETRIDLSQLGGDPKKKRKV

SEQ ID NO: 30 - DNA, 267 bp, artificial
  source 1..267: mol_type = other DNA
atgagattcccatctattttcaccgctgtcttgttcgctgcctcctctgcattggctgcccctgttaacactaccactgaagacgagactgctcaaattccagctgaagcagttatcggttactctgaccttgagggtgatttcgacgtcgctgttttgcctttctctaactccactaacaacggtttgttgttcattaacaccactatcgcttccattgctgctaaggaagagggtgtctctctcgagaagagagaggccgaagct

SEQ ID NO: 31 - DNA, 267 bp, artificial
  source 1..267: mol_type = genomic DNA
atgagattcccctccatcttcaccgctgttttgttcgctgcttcttctgctttggctgctccagttaacactactactgaggacgagactgctcagattccagctgaagctgttattggttactccgacttggaaggtgacttcgacgttgctgttttgccattctccaactccaccaacaacggtctgttgttcatcaacaccactatcgcttccattgccgctaaagaagaaggcgtttccttggagaagagagaggctgaagct

SEQ ID NO: 32 - DNA, 810 bp, artificial
  source 1..810: mol_type = genomic DNA
atgggtaaggaaaagactcacgtttcgaggccgcgattaaattccaacatggatgctgatttatatgggtataaatgggctcgcgataatgtcgggcaatcaggtgcgacaatctatcgattgtatgggaagcccgatgcgccagagttgtttctgaaacatggcaaaggtagcgttgccaatgatgttacagatgagatggtcagactaaactggctgacggaatttatgcctcttccgaccatcaagcattttatccgtactcctgatgatgcatggttactcaccactgcgatccccggcaaaacagcattccaggtattagaagaatatcctgattcaggtgaaaatattgttgatgcgctggcagtgttcctgcgccggttgcattcgattcctgtttgtaattgtccttttaacagcgatcgcgtatttcgtctggctcaggcgcaatcacgaatgaataacggtttggttgatgcgagtgattttgatgacgagcgtaatggctggcctgttgaacaagtctggaaagaaatgcataagcttttgccattctcaccggattcagtcgtcactcatggtgatttctcacttgataaccttatttttgacgaggggaaattaataggttgtattgatgttggacgagtcggaatcgcagaccgataccaggatcttgccatcctatggaactgcctcggtgagttttctccttcattacagaaacggctttttcaaaaatatggtattgataatcctgatatgaataaattgcagtttcatttgatgctcgatgagtttttctaa

SEQ ID NO: 33 - DNA, 399 bp, artificial
  source 1..399: mol_type = genomic DNA
atggccaagcctttgtctcaagaagaatccaccctcattgaaagagcaacggctacaatcaacagcatccccatctctgaagactacagcgtcgccagcgcagctctctctagcgacggccgcatcttcactggtgtcaatgtatatcattttactgggggaccttgtgcagaactcgtggtgctgggcactgctgctgctgcggcagctggcaacctgacttgtatcgtcgcgatcggaaatgagaacaggggcatcttgagcccctgcggacggtgccgacaggtgcttctcgatctgcatcctgggatcaaagccatagtgaaggacagtgatggacagccgacggcagttgggattcgtgaattgctgccctctggttatgtgtgggagggctaa

SEQ ID NO: 34 - DNA, 549 bp, artificial
  source 1..549: mol_type = other DNA
gttgtagttttaatatagtttgagtatgagatggaactcagaacgaaggaattatcaccagtttatatattctgaggaaagggtgtgtcctaaattggacagtcacgatggcaataaacgctcagccaatcagaatgcaggagccataaattgttgtattattgctgcaagatttatgtgggttcacattccactgaatggttttcactgtagaattggtgtcctagttgttatgtttcgagatgttttcaagaaaaactaaaatgcacaaactgaccaataatgtgccgtcgcgcttggtacaaacgtcaggattgccaccacttttttcgcactctggtacaaaagttcgcacttcccactcgtatgtaacgaaaaacagagcagtctatccagaacgagacaaattagcgcgtactgtcccattccataaggtatcataggaaacgagagtcctccccccatcacgtatatataaacacactgatatcccacatccgcttgtcaccaaactaatacatccagttcaagttacctaaacaaatcaaa